European Patent Application EP 4 692 339 A1, published February 11, 2026. Title: Medium composition for improving pectinase productivity of Bacillus spp. and method for producing pectinase using thereof. Applicant: CJ CheilJedang Corporation. Application KR. The sequence listing filed with the application follows.

SEQUENCE LISTING (2 sequences)

SEQ ID NO: 1 - protein, 314 aa, synthetic construct
  REGION 1..314: note = amino acid sequence of pelA enzyme
ASALNSGKVNPLADFSLKGFAALNGGTTGGEGGQTVTVTTGDQLIAALKNKNANTPLKIYVNGTITTSNTSASKIDVKDVSNVSIVGSGTKGELKGIGIKIWRANNIIIRNLKIHEVASGDKDAIGIEGPSKNIWVDHNELYHSLNVDKDYYDGLFDVKRDAEYITFSWNYVHDGWKSMLMGSSDSDNYNRTITFHHNWFENLNSRVPSFRFGEGHIYNNYFNKIIDSGINSRMGARIRIENNLFENAKDPIVSWYSSSPGYWHVSNNKFVNSRGSMPTTSTTTYNPPYSYSLDNVDNVKSIVKQNAGVGKINP

SEQ ID NO: 2 - DNA, 8682 bp, synthetic construct
  misc_feature 1..8682: note = plasmid expressing pelA
  source 1..8682: mol_type = other DNA
aattcactggccgtcgttttacaacgtcgtgactgggaaaaccctggcgttacccaacttaatcgccttgcagcacatccccctttcgccagctggcgtaatagcgaagaggcccgcaccgatcgcccttcccaacagttgcgcagcctgaatggcgaatggcgcctgatgcggtattttctccttacgcatctgtgcggtatttcacaccgcatatggtgcactctcagtacaatctgctctgatgccgcatagttaagccagccccgacacccgccaacacccgctgacgcgccctgacgggcttgtctgctcccggcatccgcttacagacaagctgtgaccgtctccgggagctgcatgtgtcagaggttttcaccgtcatcaccgaaacgcgcgagacgaaagggcctcgtgatacgcctatttttataggttaatgtcatgataataatggtttcttagacgtcaggtggcacttttcggggaaatgtgcgcggaacccctatttgtttatttttctaaatacattcaaatatgtatccgctcatgagacaataaccctgataaatgcttcaataatattgaaaaaggaagagtatgagtattcaacatttccgtgtcgcccttattcccttttttgcggcattttgccttcctgtttttgctcacccagaaacgctggtgaaagtaaaagatgctgaagatcagttgggtgcacgagtgggttacatcgaactggatctcaacagcggtaagatccttgagagttttcgccccgaagaacgttttccaatgatgagcacttttaaagttctgctatgtggcgcggtattatcccgtattgacgccgggcaagagcaactcggtcgccgcatacactattctcagaatgacttggttgagtactcaccagtcacagaaaagcatcttacggatggcatgacagtaagagaattatgcagtgctgccataaccatgagtgataacactgcggccaacttacttctgacaacgatcggaggaccgaaggagctaaccgcttttttgcacaacatgggggatcatgtaactcgccttgatcgttgggaaccggagctgaatgaagccataccaaacgacgagcgtgacaccacgatgcctgtagcaatggcaacaacgttgcgcaaactattaactggcgaactacttactctagcttcccggcaacaattaatagactggatggaggcggataaagttgcaggaccacttctgcgctcggcccttccggctggctggtttattgctgataaatctggagccggtgagcgtgggtctcgcggtatcattgcagcactggggccagatggtaagccctcccgtatcgtagttatctacacgacggggagtcaggcaactatggatgaacgaaatagacagatcgctgagataggtgcctcactgattaagcattggtaactgtcagaccaagtttactcatatatactttagattgatttaaaacttcatttttaatttaaaaggatctaggtgaagatcctttttgataatctcatgaccaaaatcccttaacgtgagttttcgttccactgagcgtcagaccccgtagaaaagatcaaaggatcttcttgagatcctttttttctgcgcgtaatctgctgcttgcaaacaaaaaaaccaccgctaccagcggtggtttgtttgccggatcaagagctaccaactctttttccgaaggtaactggcttcagcagagcgcagataccaaatactgttcttctagtgtagccgtagttaggccaccacttcaagaactctgtagcaccgcctacatacctcgctctgctaatcctgttaccagtggctgctgccagtggcgataagtcgtgtcttaccgggttggactcaagacgatagttaccggataaggcgcagcggtcgggctgaacggggggttcgtgcacacagcccagcttggagcgaacgacctacaccgaactgagatacctacagcgtgagctatgagaaagcgccacgcttcccgaagggagaaaggcggacaggtatccggtaagcggcagggtcggaacaggagagcgcacgagggagcttccagggggaaacgcctggtatctttatagtcctgtcgggtttcgccacctctgacttgagcgtcgatttttgtgatgctcgtcaggggggcggagcctatggaaaaacgccagcaacgcggcctttttacggttcctggccttttgctggccttttgctcacatgttctttcctgcgttatcccctgattctgtggataaccgtattaccgcctttgagtgagctgataccgctcgccgcagccgaacgaccgagcgcagcgagtcagtgagcgaggaagcggaagagcgcccaatacgcaaaccgcctctccccgcgcgttggccgattcattaatgcagctggcacgacaggtttcccgactggaaagcgggcagtgagcgcaacgcaattaatgtgagttagctcactcattaggcaccccaggctttacactttatgcttccggctcgtatgttgtgtggaattgtgagcggataacaatttcacacaggaaacagctatgaccatgattacgccaagcttttaaagaagtcattccttgttttttaacagcctgtgatccgcactataaagaagtgtttaccagccttagagtcgatgacggagcacccgtttttatcgtcccgtatcttttgtttaccgggcttttgatgactgagattgaacgggaagtccaaaagctacaagcggtcaatcggaatgtgcatctcgcttcatacttaggttttcacccgcatattaagcaggcgtttttgaaccgtgtgacagaagctgttcgaaaccccggcgggcggtttgattttaaggggggacagtatgctgcctcttcacattaatctcagcggaaaaagaatcatcattgctggcgggggcaatgttgcattaagaaggctgaaaacggtgcttccggaaggcgctgatattaccgtgatcagtcctgaggccctgcctgaaattaaaaagctggcggatgaaggacgcatccgctggattccccggagaattgaaatgaaagatctcaagcccgcttttttcattattgccgcgacaaatgaccgaggcgtgaatcaggagatagccgcaaacgcttctgaaacgcagctggtcaactgtgtaagcaaggctgaacaaggcagcgtatatatgccgaagatcatccgcaaagggcgcattcaagtatcagtatcaacaagcggggcaagccccgcacatacgaaaagactggctgaaaacattgagcctttgatgactgatgatttggctgaagaagtggatcgattgtttgagaaaagaagaagaccataaaaataccttgtctgtcatcagacagggtattttttatgctgtccagactgtccgctgtgtaaaaaataggaataaaggggggttgttattattttactgatatgtaaaatataatttgtataagaaaatgagagggagaggaaacatgaggagggaaccgaatgaaaaaactgatctcaatcatcttcatcttcgtacttggcgtagttggctcactgacagcagcagttagcgcagaagcagccagcgcactgaacagcggcaaagtcaacccacttgcagacttcagcctgaaaggcttcgcagcactgaacggcggcacaacaggcggcgaaggcggccaaacagttacagtcacaacaggcgaccaattaatcgcagcactgaaaaacaaaaacgccaacacaccactgaaaatctacgtcaacggcacaatcacaacaagcaacacatctgccagcaaaattgacgtcaaagatgttagcaacgtcagcattgtaggctctggcacaaaaggcgaactgaaaggcattggcatcaaaatctggcgtgccaacaacatcatcatccgtaacctgaaaattcacgaagtagctagcggcgacaaagacgccatcggcatcgaaggcccaagcaaaaacatctgggtagaccacaacgaattataccactctctgaacgtagacaaagactactacgacggcttattcgacgtcaaacgtgacgcagaatacatcacattcagctggaactacgtacatgacggctggaaaagcatgttaatgggctctagcgactctgacaactacaaccgtacaatcacattccaccacaactggttcgaaaacctgaacagccgtgtaccaagcttccgtttcggcgaaggccacatctacaacaactacttcaacaaaatcatcgacagcggcatcaacagccgtatgggcgcacgtatccgtatcgaaaacaaccttttcgaaaacgccaaagatccaatcgtcagctggtactctagctctcctggctactggcacgttagcaacaacaaattcgtcaacagccgtggctctatgccaacaacaagcacaacaacatacaacccaccatactcttacagccttgacaacgttgacaacgttaaatctatcgtcaaacaaaacgcaggcgttggcaaaatcaacccataatcaataataaggtaataaaaaaacacctccaagctgagtgcgggtatcagcttggaggtgcgtttattttttcagccgtatgacaaggtcggcatcaggtgtgacaaatacggtatgctggctgtcataggtgacaaatccgggttttgcgccgtttggctttttcacatgtctgatttttgtataatcaacaggcacggagccggaatctttcgccttggaaaaataagcggcgatcgtagctgcttccaatatggattgttcatcgggatcgctgcttttaatcacaacgtgggaccccggtatgtctcgatccagttgctcaaaaaaatctcggtcagatgttactagcaactcatttacaagaacagcatctttcctcgtttttcttgtacctgttttttgtgattcaataatttctttgacacgttcgttgtaatcaatatttttatcatttttcaaatcataattttcacgtgttcgctcatggtcaatatcatcattcgttctactttttcgctctctttgattatgaaattgcatgccttttagtccagctgatttcactttttgcattctacaaactgcataactcatatgtaaatcgctcctttttaggtggcacaaatatgaggcattttcgctctttccggcaaccacttccaagtaaagtataacacactatactttatattcataaagtgtgtgctctgcgaggctgtcggcagtgccgaccaaaaccataaaacctttaagacctttcttttttttacgagaaaaaagaaacaaaaaaacctgccctctgccacctcagcaaaggggggttttgctctcgtgctcgtttaaaaatcagcaagggacaggtagtattttttgagaagatcactcaaaaaatctccacctttaaacccttgccaatttttattttgtccgttttgtctagcttaccgaaagccagactcagcaagaataaaatttttattgtctttcggttttctagtgtaacggacaaaaccactcaaaataaaaaagatacaagagaggtctctcgtatcttttattcagcaatcgcgcccgattgctgaacagattaataatagattttagctttttatttgttgaaaaaagctaatcaaattgttgtcgggatcaattactgcaaagtctcgttcatcccaccactgatcttttaatgatgtattggggtgcaaaatgcccaaaggcttaatatgttgatataattcatcaattccctctacttcaatgcggcaactagcagtaccagcaataaacgactccgcacctgtacaaaccggtgaatcattactacgagagcgccagccttcatcacttgcctcccatagatgaatccgaacctcattacacattagaactgcgaatccatcttcatggtgaaccaaagtgaaacctagtttatcgcaataaaaacctatactctttttaatatccccgactggcaatgccgggatagactgtaacattctcacgcataaaatcccctttcattttctaatgtaaatctattaccttattattaattcaattcgctcataattaatcctttttcttattacgcaaaatggcccgatttaagcacaccctttattccgttaatgcgccatgacagccatgataattactaatactaggagaagttaataaatacgtaaccaacatgattaacaattattagaggtcatcgttcaaaatggtatgcgttttgacacatccactatatatccgtgtcgttctgtccactcctgaatcccattccagaaattctctagcgattccagaagtttctcagagtcggaaagttgaccagacattacgaactggcacagatggtcataacctgaaggaagatctgattgcttaactgcttcagttaagaccgaagcgctcgtcgtataacagatgcgatgatgcagaccaatcaacatggcacctgccattgctacctgtacagtcaaggatggtagaaatgttgtcggtccttgcacacgaatattacgccatttgcctgcatattcaaacagctcttctacgataagggcacaaatcgcatcgtggaacgtttgggcttctaccgatttagcagtttgatacactttctctaagtatccacctgaatcataaatcggcaaaatagagaaaaattgaccatgtgtaagcggccaatctgattccacctgagatgcataatctagtagaatctcttcgctatcaaaattcacttccaccttccactcaccggttgtccattcatggctgaactctgcttcctctgttgacatgacacacatcatctcaatatccgaatagggcccatcagtctgacgaccaagagagccataaacaccaatagccttaacatcatccccatatttatccaatattcgttccttaatttcatgaacaatcttcattctttcttctctagtcattattattggtccattcactattctcattcccttttcagataattttagatttgcttttctaaataagaatatttggagagcaccgttcttattcagctattaataactcgtcttcctaagcatccttcaatccttttaataacaattatagcatctaatcttcaacaaactggcccgtttgttgaactactctttaataaaataatttttccgttcccaattccacattgcaataatagaaaatccatcttcatcggctttttcgtcatcatctgtatgaatcaaatcgccttcttctgtgtcatcaaggtttaattttttatgtatttcttttaacaaaccaccataggagattaaccttttacggtgtaaaccttcctccaaatcagacaaacgtttcaaattcttttcttcatcatcggtcataaaatccgtatcctttacaggatattttgcagtttcgtcaattgccgattgtatatccgatttatatttatttttcggtcgaatcatttgaacttttacatttggatcatagtctaatttcattgcctttttccaaaattgaatccattgtttttgattaacgtagttttctgtattcttaaaataagttggttccacacataccaatacatgcatgtgctgattataagaattatctttattatttattgtcacttccgttgcacgcataaaaccaacaagatttttattaatttttttatattgcatcattcggcgaaatccttgagccatatctgacaaactcttatttaattcttcgccatcataaacatttttaactgttaatgtgagaaacaaccaacgaactgttggcttttgtttaataacttcagcaacaaccttttgtgactgaatgccatgtttcattgctctcctccagttgcacattggacaaagcctggatttacaaaaccacactcgatacaactttctttcgcctgtttcacgattttgtttatactctaatatttcagcacaatcttttactctttcagcctttttaaattcaagaatatgcagaagttcaaagtaatcaacattagcgattttcttttctctccatggtctcacttttccactttttgtcttgtccactaaaacccttgatttttcatctgaataaatgctactattaggacacataatattaaaagaaacccccatctatttagttatttgtttagtcacttataactttaacagatggggtttttctgtgcaaccaattttaagggttttcaatactttaaaacacatacataccaacacttcaacgcacctttcagcaactaaaataaaaatgacgttatttctatatgtatcaagataagaaagaacaagttcaaaaccatcaaaaaaagacaccttttcaggtgctttttttattttataaactcattccctgatctcgacttcgttctttttttacctctcggttatgagttagttcaaattcgttctttttaggttctaaatcgtgtttttcttggaattgtgctgttttatcctttaccttgtctacaaaccccttaaaaacgtttttaaaggcttttaagccgtctgtacgttccttaagg